European Patent Specification EP 3 712 264 B1, published April 10, 2024. Title: CYSTATHIONINE BETA-SYNTHASE ENZYME FOR TREATMENT OF HOMOCYSTINURIA. Applicant: The Regents of the University of Colorado Kraus, Jan P Majtan, Tomas Bublil, Erez. The sequence listing filed with the application follows.

SEQUENCE LISTING (16 sequences)

SEQ ID NO: 1 - DNA, 1656 bp, Homo sapiens
atgccttctgagaccccccaggcagaagtggggcccacaggctgcccccaccgctcagggccacactcggcgaaggggagcctggagaaggggtccccagaggataaggaagccaaggagcccctgtggatccggcccgatgctccgagcaggtgcacctggcagctgggccggcctgcctccgagtccccacatcaccacactgccccggcaaaatctccaaaaatcttgccagatattctgaagaaaatcggggacacccctatggtcagaatcaacaagattgggaagaagttcggcctgaagtgtgagctcttggccaagtgtgagttcttcaacgcgggcgggagcgtgaaggaccgcatcagcctgcggatgattgaggatgctgagcgcgacgggacgctgaagcccggggacacgattatcgagccgacatccgggaacaccgggatcgggctggccctggctgcggcagtgaggggctatcgctgcatcatcgtgatgccagagaagatgagctccgagaaggtggacgtgctgcgggcactgggggctgagattgtgaggacgcccaccaatgccaggttcgactccccggagtcacacgtgggggtggcctggcggctgaagaacgaaatccccaattctcacatcctagaccagtaccgcaacgccagcaaccccctggctcactacgacaccaccgctgatgagatcctgcagcagtgtgatgggaagctggacatgctggtggcttcagtgggcacgggcggcaccatcacgggcattgccaggaagctgaaggagaagtgtcctggatgcaggatcattggggtggatcccgaagggtccatcctcgcagagccggaggagctgaaccagacggagcagacaacctacgaggtggaagggatcggctacgacttcatccccacggtgctggacaggacggtggtggacaagtggttcaagagcaacgatgaggaggcgttcacctttgcccgcatgctgatcgcgcaagaggggctgctgtgcggtggcagtgctggcagcacggtggcggtggccgtgaaggctgcgcaggagctgcaggagggccagcgctgcgtggtcattctgcccgactcagtgcggaactacatgaccaagttcctgagcgacaggtggatgctgcagaagggctttctgaaggaggaggacctcacggagaagaagccctggtggtggcacctccgtgttcaggagctgggcctgtcagccccgctgaccgtgctcccgaccatcacctgtgggcacaccatcgagatcctccgggagaagggcttcgaccaggcgcccgtggtggatgaggcgggggtaatcctgggaatggtgacgcttgggaacatgctctcgtccctgcttgccgggaaggtgcagccgtcagaccaagttggcaaagtcatctacaagcagttcaaacagatccgcctcacggacacgctgggcaggctctcgcacatcctggagatggaccacttcgccctggtggtgcacgagcagatccagtaccacagcaccgggaagtccagtcagcggcagatggtgttcggggtggtcaccgccattgacttgctgaacttcgtggccgcccaggagcgggaccagaagtga

SEQ ID NO: 2 - protein, 551 aa, Homo sapiens
MPSETPQAEVGPTGCPHRSGPHSAKGSLEKGSPEDKEAKEPLWIRPDAPSRCTWQLGRPASESPHHHTAPAKSPKILPDILKKIGDTPMVRINKIGKKFGLKCELLAKCEFFNAGGSVKDRISLRMIEDAERDGTLKPGDTIIEPTSGNTGIGLALAAAVRGYRCIIVMPEKMSSEKVDVLRALGAEIVRTPTNARFDSPESHVGVAWRLKNEIPNSHILDQYRNASNPLAHYDTTADEILQQCDGKLDMLVASVGTGGTITGIARKLKEKCPGCRIIGVDPEGSILAEPEELNQTEQTTYEVEGIGYDFIPTVLDRTVVDKWFKSNDEEAFTFARMLIAQEGLLCGGSAGSTVAVAVKAAQELQEGQRCVVILPDSVRNYMTKFLSDRWMLQKGFLKEEDLTEKKPWWWHLRVQELGLSAPLTVLPTITCGHTIEILREKGFDQAPVVDEAGVILGMVTLGNMLSSLLAGKVQPSDQVGKVIYKQFKQIRLTDTLGRLSHILEMDHFALVVHEQIQYHSTGKSSQRQMVFGVVTAIDLLNFVAAQERDQK

SEQ ID NO: 3 - protein, 413 aa, Artificial Sequence
  Synthetic
MPSETPQAEVGPTGCPHRSGPHSAKGSLEKGSPEDKEAKEPLWIRPDAPSRCTWQLGRPASESPHHHTAPAKSPKILPDILKKIGDTPMVRINKIGKKFGLKCELLAKCEFFNAGGSVKDRISLRMIEDAERDGTLKPGDTIIEPTSGNTGIGLALAAAVRGYRCIIVMPEKMSSEKVDVLRALGAEIVRTPTNARFDSPESHVGVAWRLKNEIPNSHILDQYRNASNPLAHYDTTADEILQQCDGKLDMLVASVGTGGTITGIARKLKEKCPGCRIIGVDPEGSILAEPEELNQTEQTTYEVEGIGYDFIPTVLDRTVVDKWFKSNDEEAFTFARMLIAQEGLLCGGSAGSTVAVAVKAAQELQEGQRCVVILPDSVRNYMTKFLSDRWMLQKGFLKEEDLTEKKPWWWHLR

SEQ ID NO: 4 - DNA, 1242 bp, Artificial Sequence
  Synthetic
atgccgtcagaaaccccgcaggcagaagtgggtccgacgggttgcccgcaccgtagcggtccgcattctgcaaaaggcagtctggaaaaaggttccccggaagataaagaagccaaagaaccgctgtggattcgtccggacgcaccgtcacgctgtacctggcagctgggtcgtccggcaagcgaatctccgcatcaccatacggctccggcgaaaagtccgaaaattctgccggatatcctgaagaaaattggtgacaccccgatggttcgtatcaacaaaatcggcaaaaaattcggtctgaaatgcgaactgctggctaaatgtgaatttttcaatgcgggcggttccgtgaaagatcgtatctcactgcgcatgattgaagatgctgaacgcgacggcaccctgaaaccgggtgatacgattatcgaaccgacctctggcaacacgggtatcggtctggcactggcggcggcagtccgtggttatcgctgcattatcgtgatgccggaaaaaatgagctctgaaaaagttgatgtcctgcgtgctctgggcgcggaaattgttcgtaccccgacgaatgcccgcttcgacagtccggaatcccatgtgggtgttgcatggcgcctgaaaaacgaaatcccgaattcgcacattctggatcagtatcgtaacgctagcaatccgctggcgcattacgataccacggccgacgaaatcctgcagcaatgtgatggcaaactggacatgctggtcgcttctgtgggtaccggcggtaccattacgggcatcgcgcgtaaactgaaagaaaaatgcccgggctgtcgcattatcggtgtggatccggaaggcagtattctggcggaaccggaagaactgaaccagaccgaacaaaccacgtatgaagttgaaggcatcggttacgattttattccgaccgtcctggatcgcacggtggttgacaaatggttcaaaagcaatgacgaagaagcctttaccttcgcacgtatgctgatcgctcaggaaggtctgctgtgcggtggttcagcaggttcgacggtcgcagtggcagttaaagctgcgcaggaactgcaagaaggtcaacgttgtgtcgtgattctgccggattctgttcgcaactacatgaccaaatttctgagtgaccgttggatgctgcaaaaaggcttcctgaaagaagaagatctgaccgagaaaaaaccgtggtggtggcacctgcgctaa

SEQ ID NO: 5 - DNA, 30 bp, Artificial Sequence
  Synthetic oligonucleotide
cgtagaattcacctttgcccgcatgctgat

SEQ ID NO: 6 - DNA, 35 bp, Artificial Sequence
  Synthetic oligonucleotide
tacgggtacctcaacggaggtgccaccaccagggc

SEQ ID NO: 7 - DNA, 29 bp, Artificial Sequence
  Synthetic oligonucleotide
agtcgcccatggcgtcagaaaccccgcag

SEQ ID NO: 8 - DNA, 31 bp, Artificial Sequence
  Synthetic oligonucleotide
atcgcgctcgagttagcgcaggtgccaccac

SEQ ID NO: 9 - DNA, 30 bp, Artificial Sequence
  Synthetic oligonucleotide
ggagatataccatgccgtcagaaaccccgc

SEQ ID NO: 10 - DNA, 30 bp, Artificial Sequence
  Synthetic oligonucleotide
gcggggtttctgacggcatggtatatctcc

SEQ ID NO: 11 - DNA, 23 bp, Artificial Sequence
  Synthetic oligonucleotide
tgggtccgacgggtagcccgcac

SEQ ID NO: 12 - DNA, 23 bp, Artificial Sequence
  Synthetic oligonucleotide
gtgcgggctacccgtcggaccca

SEQ ID NO: 13 - protein, 413 aa, Artificial Sequence
  Truncated human C15S mutant CBS polypeptide
MPSETPQAEVGPTGSPHRSGPHSAKGSLEKGSPEDKEAKEPLWIRPDAPSRCTWQLGRPASESPHHHTAPAKSPKILPDILKKIGDTPMVRINKIGKKFGLKCELLAKCEFFNAGGSVKDRISLRMIEDAERDGTLKPGDTIIEPTSGNTGIGLALAAAVRGYRCIIVMPEKMSSEKVDVLRALGAEIVRTPTNARFDSPESHVGVAWRLKNEIPNSHILDQYRNASNPLAHYDTTADEILQQCDGKLDMLVASVGTGGTITGIARKLKEKCPGCRIIGVDPEGSILAEPEELNQTEQTTYEVEGIGYDFIPTVLDRTVVDKWFKSNDEEAFTFARMLIAQEGLLCGGSAGSTVAVAVKAAQELQEGQRCVVILPDSVRNYMTKFLSDRWMLQKGFLKEEDLTEKKPWWWHLR

SEQ ID NO: 14 - DNA, 1242 bp, Artificial Sequence
  Truncated human C15S mutant CBS Nucleotide
atgccgtcagaaaccccgcaggcagaagtgggtccgacgggtagcccgcaccgtagcggtccgcattctgcaaaaggcagtctggaaaaaggttccccggaagataaagaagccaaagaaccgctgtggattcgtccggacgcaccgtcacgctgtacctggcagctgggtcgtccggcaagcgaatctccgcatcaccatacggctccggcgaaaagtccgaaaattctgccggatatcctgaagaaaattggtgacaccccgatggttcgtatcaacaaaatcggcaaaaaattcggtctgaaatgcgaactgctggctaaatgtgaatttttcaatgcgggcggttccgtgaaagatcgtatctcactgcgcatgattgaagatgctgaacgcgacggcaccctgaaaccgggtgatacgattatcgaaccgacctctggcaacacgggtatcggtctggcactggcggcggcagtccgtggttatcgctgcattatcgtgatgccggaaaaaatgagctctgaaaaagttgatgtcctgcgtgctctgggcgcggaaattgttcgtaccccgacgaatgcccgcttcgacagtccggaatcccatgtgggtgttgcatggcgcctgaaaaacgaaatcccgaattcgcacattctggatcagtatcgtaacgctagcaatccgctggcgcattacgataccacggccgacgaaatcctgcagcaatgtgatggcaaactggacatgctggtcgcttctgtgggtaccggcggtaccattacgggcatcgcgcgtaaactgaaagaaaaatgcccgggctgtcgcattatcggtgtggatccggaaggcagtattctggcggaaccggaagaactgaaccagaccgaacaaaccacgtatgaagttgaaggcatcggttacgattttattccgaccgtcctggatcgcacggtggttgacaaatggttcaaaagcaatgacgaagaagcctttaccttcgcacgtatgctgatcgctcaggaaggtctgctgtgcggtggttcagcaggttcgacggtcgcagtggcagttaaagctgcgcaggaactgcaagaaggtcaacgttgtgtcgtgattctgccggattctgttcgcaactacatgaccaaatttctgagtgaccgttggatgctgcaaaaaggcttcctgaaagaagaagatctgaccgagaaaaaaccgtggtggtggcacctgcgctaa

SEQ ID NO: 15 - DNA, 1656 bp, Artificial Sequence
  Full length human C15S mutant CBS nucleotide
atgccgtcagaaaccccgcaggcagaagtgggtccgacgggtagcccgcaccgtagcggtccgcattctgcaaaaggcagtctggaaaaaggttccccggaagataaagaagccaaagaaccgctgtggattcgtccggacgcaccgtcacgctgtacctggcagctgggtcgtccggcaagcgaatctccgcatcaccatacggctccggcgaaaagtccgaaaattctgccggatatcctgaagaaaattggtgacaccccgatggttcgtatcaacaaaatcggcaaaaaattcggtctgaaatgcgaactgctggctaaatgtgaatttttcaatgcgggcggttccgtgaaagatcgtatctcactgcgcatgattgaagatgctgaacgcgacggcaccctgaaaccgggtgatacgattatcgaaccgacctctggcaacacgggtatcggtctggcactggcggcggcagtccgtggttatcgctgcattatcgtgatgccggaaaaaatgagctctgaaaaagttgatgtcctgcgtgctctgggcgcggaaattgttcgtaccccgacgaatgcccgcttcgacagtccggaatcccatgtgggtgttgcatggcgcctgaaaaacgaaatcccgaattcgcacattctggatcagtatcgtaacgctagcaatccgctggcgcattacgataccacggccgacgaaatcctgcagcaatgtgatggcaaactggacatgctggtcgcttctgtgggtaccggcggtaccattacgggcatcgcgcgtaaactgaaagaaaaatgcccgggctgtcgcattatcggtgtggatccggaaggcagtattctggcggaaccggaagaactgaaccagaccgaacaaaccacgtatgaagttgaaggcatcggttacgattttattccgaccgtcctggatcgcacggtggttgacaaatggttcaaaagcaatgacgaagaagcctttaccttcgcacgtatgctgatcgctcaggaaggtctgctgtgcggtggttcagcaggttcgacggtcgcagtggcagttaaagctgcgcaggaactgcaagaaggtcaacgttgtgtcgtgattctgccggattctgttcgcaactacatgaccaaatttctgagtgaccgttggatgctgcaaaaaggcttcctgaaagaagaagatctgaccgagaaaaaaccgtggtggtggcacctgcgcgtgcaggaactgggtctgtccgcaccgctgaccgttctgccgaccatcacgtgcggccatacgattgaaatcctgcgtgaaaaaggttttgatcaggccccggttgtcgacgaagcaggcgtgattctgggtatggttaccctgggtaacatgctgagttccctgctggcgggcaaagtgcaaccgagcgatcaggttggtaaagtcatctacaaacaattcaaacagattcgtctgaccgatacgctgggccgcctgtcgcacatcctggaaatggaccatttcgcgctggttgtgcacgaacagattcaataccatagcaccggcaaatcatcgcagcgccaaatggtctttggtgtcgtgacggccattgatctgctgaatttcgtggccgcacaagaacgtgaccagaaataa

SEQ ID NO: 16 - protein, 551 aa, Artificial Sequence
  Full length human C15S mutant CBS polypeptide
MPSETPQAEVGPTGSPHRSGPHSAKGSLEKGSPEDKEAKEPLWIRPDAPSRCTWQLGRPASESPHHHTAPAKSPKILPDILKKIGDTPMVRINKIGKKFGLKCELLAKCEFFNAGGSVKDRISLRMIEDAERDGTLKPGDTIIEPTSGNTGIGLALAAAVRGYRCIIVMPEKMSSEKVDVLRALGAEIVRTPTNARFDSPESHVGVAWRLKNEIPNSHILDQYRNASNPLAHYDTTADEILQQCDGKLDMLVASVGTGGTITGIARKLKEKCPGCRIIGVDPEGSILAEPEELNQTEQTTYEVEGIGYDFIPTVLDRTVVDKWFKSNDEEAFTFARMLIAQEGLLCGGSAGSTVAVAVKAAQELQEGQRCVVILPDSVRNYMTKFLSDRWMLQKGFLKEEDLTEKKPWWWHLRVQELGLSAPLTVLPTITCGHTIEILREKGFDQAPVVDEAGVILGMVTLGNMLSSLLAGKVQPSDQVGKVIYKQFKQIRLTDTLGRLSHILEMDHFALVVHEQIQYHSTGKSSQRQMVFGVVTAIDLLNFVAAQERDQK